European Patent Application EP 4 600 367 A1, published August 13, 2025. Title: Enzymatische Spaltung von N-Alkylverbindungen nach der Chemolyse von Polyurethanen. Applicant: Covestro Deutschland AG. Application EP. The sequence listing filed with the application follows.

SEQUENCE LISTING (5 sequences)

SEQ ID NO: 1 - protein, 495 aa, Aspergillus niger
MTSRDGYQWTPETGLTQGVPSLGVISPPTNIEDTDKDGPWDVIVIGGGYCGLTATRDLTVAGFKTLLLEARDRIGGRSWSSNIDGYPYEMGGTWVHWHQSHVWREITRYKMHNALSPSFNFSRGVNHFQLRTNPTTSTYMTHEAEDELLRSALHKFTNVDGTNGRTVLPFPHDMFYVPEFRKYDEMSYSERIDQIRDELSLNERSSLEAFILLCSGGTLENSSFGEFLHWWAMSGYTYQGCMDCLISYKFKDGQSAFARRFWEEAAGTGRLGYVFGCPVRSVVNERDAARVTARDGREFAAKRLVCTIPLNVLSTIQFSPALSTERISAMQAGHVNMCTKVHAEVDNKDMRSWTGIAYPFNKLCYAIGDGTTPAGNTHLVCFGTDANHIQPDEDVRETLKAVGQLAPGTFGVKRLVFHNWVKDEFAKGAWFFSRPGMVSECLQGLREKHRGVVFANSDWALGWRSFIDGAIEEGTRAARVVLEELGTKREVKARL

SEQ ID NO: 2 - protein, 495 aa, Aspergillus niger
MTSRDGYQWTPETGLTQGVPSLGVISPPTNIEDTDKDGPWDVIVIGGGYCGLTATRDLTVAGFKTLLLEARDRIGGRSWSSNIDGYPYEMGGTWVHWHQSHVWREITRYKMHNALSPSFNFSRGVNHFQLRTNPTTSTYMTHEAEDELLRSALHKFTNVDGTNGRTVLPFPHDMFYVPEFRKYDEMSYSERIDQIRDELSLNERSSLEAFILLCSGGTLENSSFGEFLHWWAMSGYTYQGCMDCLMSYKFKDGQSAFARRFWEEAAGTGRLGYVFGCPVRSVVNERDAARVTARDGREFAAKRLVCTIPLNVLSTIQFSPALSTERISAMQAGHVSMCTKVHAEVDNKDMRSWTGIAYPFNKLCYAIGDGTTPAGNTHLVCFGNSANHIQPDEDVRETLKAVGQLAPGTFGVKRLVFHNWVKDEFAKGAWFFSRPGMVSECLQGLREKHRGVVFANSDWALGWRSFIDGAIEEGTRAARVVLEELGTKREVKARL

SEQ ID NO: 3 - protein, 488 aa, Brevibacterium oxydans
MCRSRQAARSKREESALTHLNTYESVTPDPDVDVIIIGAGISGSAAAKALHDQGASVLVVEANDRIGGRTWTEQEGAPGGPIDYGGMFIGETHTHLIELGTSLGLEMTPSGKPGDDTYIVAGNVLRAPDDQLDPNLPFVPEFLSSLKALDELADSVGWDQPWASPNAAALDSKTVATWLAETIESEEVRRLHTVIVNTLLGADPYEVSLLYWAYYVSECEGIQSAMGTRDGAQWAWWFGGAAQVSWRIADAIGRDKFLLEWPVDRIEHDESGVTLFSGQRSLRARHIVIAMSPLAANQIRFEPALPTSRAQLQARAPMGRYYKVQARYPSSFWVEQGYSGALLDTEDVGVFLLDGTKPTDTLATLIGFIGGSNYDRWAAHTPQERERAFLDLLVKAFGPQAADPSYFHETDWTQQEWAKGGPVTYMPPGVLANFGAALRDPVGKVHFAGTEASFQWSGYMEGGVRAGQKAAAAIAEELERTANKGALV

SEQ ID NO: 4 - protein, 488 aa, Brevibacterium oxydans
MCRSRQAARSKREESALTHLNTYESVTPDPDVDVIIIGAGISGSAAAKALHDQGASVLVVEANDRIGGRTWTEQEGAPGGPIDYGGMFIGETHTHLIELGTSLGLEMTPSGKPGDDTYIVAGNVLRAPDDQLDPNLPFVPEFLSSLKALDELADSVGWDQPWASPNAAALDSKTVATWLAETIESEEVRRLHTVIVNTLLGADPYEVSLLYWAYYVSECEGIQSLTGTRDGAQWAWWFGGAAQVSWRIADAIGRDKFLLEWPVDRIEHDESGVTLFSGQRSLRARHIVIAMSPLAANQIRFEPALPTSRAQLQARAPMGRIYKVQARYPSSFWVEQGYSGALLDTEDVGVFLLDGTKPTDTLATLIGFIGGSNYDRWAAHTPQERERAFLDLLVKAFGPQAADPSYFHETDWTQQEWAKGGPVTYMPPGVLANFGAALRDPVGKVHFAGTEASFQWSGYMEGGVRAGQKAAAAIAEELERTANKGALV

SEQ ID NO: 5 - protein, 460 aa, Acinetobacter sp.
MSVNDNRESASYDADVIVVGAGPSGSYAAKLLHDRGISVKLVEAKDRVGGRTWSSKTEAQGGPIDFGGQWIGETHVLLPELGEELGLETVSSIKPGNDIFVFNGQVTVGEEDQAPASASWTAELTRSFELLDEAGARLGWEAPWASPAVEALDGMTVAQWLDENVSSDEVRMIHEVMVNILNGANTTEVSMAYWAYFVHQGEGIESLIGTRSGAQIAWFVGGMGQVTELIADRLGDNLHLNWPVTSIEQQDSGVVVSSGDRRLTAKYVILATPPSDASRMIFDQPLPAKRAQLQARAPMGRLAKIQVRYRDAFWQEENLSGAAFVCGDLAFWVFDGSKPSDSLATIVGFIGGKHLDLWHSFTPEEREARFIDMLVTNIGEKARDTVYYHETDWTEQPWTGGAPVTFMPTGLLSSSGSALRGSAGRIHFAGTEAAPMWSGYIEGALRAGKIAATDIIARLG